European Patent Application EP 4 596 580 A1, published August 6, 2025. Title: ANTIBODIES SPECIFICALLY RECOGNIZING LIGHT AND USES THEREOF. Applicant: STAIDSON (BEIJING) BIOPHARMACEUTICALS CO., LTD. Application CN. The sequence listing filed with the application follows.

SEQUENCE LISTING (99 sequences)

SEQ ID NO: 1 - protein, 5 aa, synthetic construct
GYFIN

SEQ ID NO: 2 - protein, 5 aa, synthetic construct
GYFMN

SEQ ID NO: 3 - protein, 5 aa, synthetic construct
NYYVY

SEQ ID NO: 4 - protein, 5 aa, synthetic construct
NYGMN

SEQ ID NO: 5 - protein, 5 aa, synthetic construct
TYYMY

SEQ ID NO: 6 - protein, 5 aa, synthetic construct
DHIMN

SEQ ID NO: 7 - protein, 5 aa, synthetic construct
SYNVH

SEQ ID NO: 8 - protein, 17 aa, synthetic construct
RIYPYNVNTFYNQNFKG

SEQ ID NO: 9 - protein, 17 aa, synthetic construct
RIYPYNVDTFYNQNFKG

SEQ ID NO: 10 - protein, 17 aa, synthetic construct
RIYPYSGDTFYNQKFNN

SEQ ID NO: 11 - protein, 17 aa, synthetic construct
EINPTNGDPNFNEKFKS

SEQ ID NO: 12 - protein, 17 aa, synthetic construct
WINTYTGEPTYADDFKG

SEQ ID NO: 13 - protein, 17 aa, synthetic construct
EINPTNGGTIFNEKFKT

SEQ ID NO: 14 - protein, 17 aa, synthetic construct
RIYPVSGETNYNQKFMG

SEQ ID NO: 15 - protein, 17 aa, synthetic construct
AVYPGNGDTSYNQKFKG

SEQ ID NO: 16 - protein, 13 aa, synthetic construct
GTHYYGSSGAMDY

SEQ ID NO: 17 - protein, 15 aa, synthetic construct
SEHFGRNYGTGAVDY

SEQ ID NO: 18 - protein, 11 aa, synthetic construct
SNWDYGNAMDF

SEQ ID NO: 19 - protein, 10 aa, synthetic construct
DNWDGKGMDY

SEQ ID NO: 20 - protein, 10 aa, synthetic construct
GNWPYWSFDV

SEQ ID NO: 21 - protein, 10 aa, synthetic construct
GSYYWNAMDY

SEQ ID NO: 22 - protein, 12 aa, synthetic construct
GSYYYTSSYFDH

SEQ ID NO: 23 - protein, 11 aa, synthetic construct
KASQNVGTAVA

SEQ ID NO: 24 - protein, 16 aa, synthetic construct
RSSQGLVHSNGNTYLH

SEQ ID NO: 25 - protein, 16 aa, synthetic construct
RSSQSLVHSNGNTYLH

SEQ ID NO: 26 - protein, 15 aa, synthetic construct
KASQSVDFDGDGYMN

SEQ ID NO: 27 - protein, 11 aa, synthetic construct
KASQDVDTAVA

SEQ ID NO: 28 - protein, 15 aa, synthetic construct
KASQSVDFDGDNYMN

SEQ ID NO: 29 - protein, 15 aa, synthetic construct
KASQSVDFDGDSYMN

SEQ ID NO: 30 - protein, 7 aa, synthetic construct
SASNRYT

SEQ ID NO: 31 - protein, 7 aa, synthetic construct
KVSNRFS

SEQ ID NO: 32 - protein, 7 aa, synthetic construct
KASHLDS

SEQ ID NO: 33 - protein, 7 aa, synthetic construct
WASTRHT

SEQ ID NO: 34 - protein, 7 aa, synthetic construct
AASNLDS

SEQ ID NO: 35 - protein, 7 aa, synthetic construct
SASNLES

SEQ ID NO: 36 - protein, 7 aa, synthetic construct
TASNLES

SEQ ID NO: 37 - protein, 9 aa, synthetic construct
QQYSSYPYT

SEQ ID NO: 38 - protein, 9 aa, synthetic construct
SQSTHVPYT

SEQ ID NO: 39 - protein, 9 aa, synthetic construct
SQSTHVPLT

SEQ ID NO: 40 - protein, 9 aa, synthetic construct
QQSIEDPLT

SEQ ID NO: 41 - protein, 9 aa, synthetic construct
QQSIEDPFT

SEQ ID NO: 42 - protein, 9 aa, synthetic construct
HQYGSYPLT

SEQ ID NO: 43 - protein, 9 aa, synthetic construct
QQSIEDPWT

SEQ ID NO: 44 - protein, 9 aa, synthetic construct
QQSYEDPFT

SEQ ID NO: 45 - protein, 17 aa, synthetic construct
  VARIANT 8: note = X is D or N
RIYPYNVXTFYNQNFKG

SEQ ID NO: 46 - protein, 122 aa, synthetic construct
QVQLKQSGAELVRPGTSVKVSCKASGYSFTGYFINWVKQSHGKSLEWIGRIYPYNVNTFYNQNFKGRATLTADKSSSTAHMELLSLTSEDSAVYYCGRGTHYYGSSGAMDYWGQGTSVTVSS

SEQ ID NO: 47 - protein, 122 aa, synthetic construct
QVQLVQSGAEVKKPGASVKVSCKASGYSFTGYFINWVRQAPGQSLEWIGRIYPYNVNTFYNQNFKGRATLTADKSTSTAYMELSSLRSEDTAVYYCGRGTHYYGSSGAMDYWGQGTLVTVSS

SEQ ID NO: 48 - protein, 122 aa, synthetic construct
QVQLVQSGAEVKKPGASVKVSCKASGYSFTGYFINWVRQAPGQGLEWIGRIYPYNVNTFYNQNFKGRATLTADKSTSTAYMELSSLRSEDTAVYYCGRGTHYYGSSGAMDYWGQGTLVTVSS

SEQ ID NO: 49 - protein, 122 aa, synthetic construct
QVQLVQSGAEVKKPGASVKVSCKASGYSFTGYFINWVRQAPGQGLEWIGRIYPYNVNTFYNQNFKGRATMTADKSTSTAYMELSSLRSEDTAVYYCGRGTHYYGSSGAMDYWGQGTLVTVSS

SEQ ID NO: 50 - protein, 122 aa, synthetic construct
QVQLVQSGAEVKKPGASVKVSCKASGYSFTGYFINWVRQAPGQGLEWIGRIYPYNVNTFYNQNFKGRVTMTADKSTSTAYMELSSLRSEDTAVYYCGRGTHYYGSSGAMDYWGQGTLVTVSS

SEQ ID NO: 51 - protein, 122 aa, synthetic construct
QVQLVQSGAEVKKPGASVKVSCKASGYSFTGYFINWVRQAPGQGLEWIGRIYPYNVDTFYNQNFKGRVTMTADKSTSTAYMELSSLRSEDTAVYYCGRGTHYYGSSGAMDYWGQGTLVTVSS

SEQ ID NO: 52 - protein, 122 aa, synthetic construct
QVQLVQSGAEVKKPGASVKVSCKASGYSFTGYFINWVRQAPGQSLEWIGRIYPYNVDTFYNQNFKGRATLTADKSTSTAYMELSSLRSEDTAVYYCGRGTHYYGSSGAMDYWGQGTLVTVSS

SEQ ID NO: 53 - protein, 122 aa, synthetic construct
QVQLVQSGAEVKKPGASVKVSCKASGYSFTGYFINWVRQAPGQGLEWIGRIYPYNVDTFYNQNFKGRATMTADKSTSTAYMELSSLRSEDTAVYYCGRGTHYYGSSGAMDYWGQGTLVTVSS

SEQ ID NO: 54 - protein, 124 aa, synthetic construct
QVQLQQSGPELVKPGASVKISCKASGYSFTGYFMNWVKQSHGKSLEWIGRIYPYSGDTFYNQKFNNKATLTVDKSSSTAHLELLSLTSEDSAVYYCGRSEHFGRNYGTGAVDYWGQGTSVTVSS

SEQ ID NO: 55 - protein, 124 aa, synthetic construct
EVKLLESGPELVKPGASVKISCKASGYSFTGYFMNWVKQSHGKSLEWIGRIYPYSGDTFYNQKFNNKATLTVDKSSSTAHLELLSLTSEDSAVYYCGRSEHFGRNYGTGAVDYWGQGTSVTVSS

SEQ ID NO: 56 - protein, 120 aa, synthetic construct
QVQLKQSGAELVKPGASVRLSCKTSGYTFTNYYVYWVKQRPGQGLEWIGEINPTNGDPNFNEKFKSKATLTVDKSSSTAYMHLSSLTSEDSAVYYCTRSNWDYGNAMDFWGQGTSVTVSS

SEQ ID NO: 57 - protein, 120 aa, synthetic construct
EVKLEESGAELVKPGASVRLSCKTSGYTFTNYYVYWVKQRPGQGLEWIGEINPTNGDPNFNEKFKSKATLTVDKSSSTAYMHLSSLTSEDSAVYYCTRSNWDYGNAMDFWGQGTSVTVSS

SEQ ID NO: 58 - protein, 119 aa, synthetic construct
QIQLLQSGPELEKPGETVKISCKASGYTFTNYGMNWVKQAPGKGLKWMGWINTYTGEPTYADDFKGRFAFSLETSASTAYLQINNLKNEDTATYFCARDNWDGKGMDYWGQGTSVTVSS

SEQ ID NO: 59 - protein, 119 aa, synthetic construct
EVQLQQSGAELVKPGASVKLSCKASGYTFATYYMYWVKQRPGQGLEWIGEINPTNGGTIFNEKFKTKATLTVDKSSSTAYMQLSSLTSEDSAVYYCARGNWPYWSFDVWGAGTSVTVSS

SEQ ID NO: 60 - protein, 119 aa, synthetic construct
QVQLQQSGAEMASPGASVTLSCKASGYTFIDHIMNWVKKRPGQGLEWIGRIYPVSGETNYNQKFMGKATFSVDRSSSTVYMVLNSLTSEDPAVYYCGRGSYYWNAMDYWGQGTTLTVSS

SEQ ID NO: 61 - protein, 121 aa, synthetic construct
EVQLQQSGAELVKPGASVKMSCKASGYTFTSYNVHWVKQTPGQGLEWIGAVYPGNGDTSYNQKFKGKATLTADKSSNTAYMQLSSLTSEDSAVYYCARGSYYYTSSYFDHWGQGTTLTVSS

SEQ ID NO: 62 - protein, 107 aa, synthetic construct
DILLTQSHKFMSTSVGDRVSITCKASQNVGTAVAWYQQKPGQSPKLLIYSASNRYTGVPDRFTGSGSGTDFTLTISNMQSEDLADYFCQQYSSYPYTFGGGTKLEIK

SEQ ID NO: 63 - protein, 107 aa, synthetic construct
EIVLTQSPATLSVSPGERATLSCKASQNVGTAVAWYQQKPGQSPRLLIYSASNRYTGIPARFSGSGSGTEFTLTISSLQSEDFAVYFCQQYSSYPYTFGGGTKVEIK

SEQ ID NO: 64 - protein, 107 aa, synthetic construct
EIVMTQSPATLSVSPGERATLSCKASQNVGTAVAWYQQKPGQSPRLLIYSASNRYTGIPARFSGSGSGTEFTLTISSLQSEDFAVYFCQQYSSYPYTFGGGTKVEIK

SEQ ID NO: 65 - protein, 107 aa, synthetic construct
EIVLTQSPATLSVSPGERATLSCKASQNVGTAVAWYQQKPGQSPRLLIYSASNRYTGIPARFSGSGSGTEFTLTISSLQSEDFAVYYCQQYSSYPYTFGGGTKVEIK

SEQ ID NO: 66 - protein, 112 aa, synthetic construct
DVVMTQTPLSLPVSLGDQASISCRSSQGLVHSNGNTYLHWYLQKPGQSPKLLIYKVSNRFSGVPDRFSGSGSGTDFTLKISRVEAEDLGIYFCSQSTHVPYTFGGGTKLEIK

SEQ ID NO: 67 - protein, 112 aa, synthetic construct
DIVLTQSPLSLPVSLGDQASISCRSSQSLVHSNGNTYLHWYLQKPGQSPKLLIYKVSNRFSGVPDRFSGSGSGTDFTLKISRVEAEDLGVYFCSQSTHVPLTFGDGTRLEIK

SEQ ID NO: 68 - protein, 111 aa, synthetic construct
DIVMTQSPASLAVSLGQRATISCKASQSVDFDGDGYMNWYQQKPGQPPKLLIYKASHLDSGIPARFSGSGSGTDFTLNIHPVEEEDAATYYCQQSIEDPLTFGDGTRLEIK

SEQ ID NO: 69 - protein, 111 aa, synthetic construct
DIVMTQSPASLAVSLGQRATISCKASQSVDFDGDGYMNWYQQKPGQPPKLLIYKASHLDSGIPARFSASGSGTDFTLNIHPVEEEDAATYYCQQSIEDPFTFGSGTKLEIK

SEQ ID NO: 70 - protein, 107 aa, synthetic construct
DIVLTQSPKFMSTSVGDRVSITCKASQDVDTAVAWYQQKPGHSPKLLLYWASTRHTGVPDRFTGSGSGTDFTLTISNVQSEDLADYFCHQYGSYPLTFGAGTKLELK

SEQ ID NO: 71 - protein, 111 aa, synthetic construct
DIVLTQSPASLAVSLGQRATISCKASQSVDFDGDNYMNWYQQKPGQPPKLLIYAASNLDSGIPARFSASGSGTDFTLNIHPVEEEDAATYYCQQSIEDPWTFGGGTKLEIK

SEQ ID NO: 72 - protein, 111 aa, synthetic construct
DIVMTQSPASLAVSLGQRATISCKASQSVDFDGDSYMNWYQQKPGQPPKLLIYSASNLESGIPARFSGSGSGTDFTLNIHPVEEEDAATYYCQQSIEDPWTFGGGTKLEIK

SEQ ID NO: 73 - protein, 111 aa, synthetic construct
DIVLTQSPASLAVSLGQRATISCKASQSVDFDGDSYMNWYQQKPGQPPKLLIYTASNLESGIPARFTGSGSGTDFTLNIHPVEEEDAATYYCQQSYEDPFTFGSGTKLEIK

SEQ ID NO: 74 - protein, 330 aa, synthetic construct
ASTKGPSVFPLAPSSKSTSGGTAALGCLVKDYFPEPVTVSWNSGALTSGVHTFPAVLQSSGLYSLSSVVTVPSSSLGTQTYICNVNHKPSNTKVDKKVEPKSCDKTHTCPPCPAPELLGGPSVFLFPPKPKDTLMISRTPEVTCVVVDVSHEDPEVKFNWYVDGVEVHNAKTKPREEQYNSTYRVVSVLTVLHQDWLNGKEYKCKVSNKALPAPIEKTISKAKGQPREPQVYTLPPSREEMTKNQVSLTCLVKGFYPSDIAVEWESNGQPENNYKTTPPVLDSDGSFFLYSKLTVDKSRWQQGNVFSCSVMHEALHNHYTQKSLSLSPGK

SEQ ID NO: 75 - protein, 327 aa, synthetic construct
ASTKGPSVFPLAPCSRSTSESTAALGCLVKDYFPEPVTVSWNSGALTSGVHTFPAVLQSSGLYSLSSVVTVPSSSLGTKTYTCNVDHKPSNTKVDKRVESKYGPPCPSCPAPEFLGGPSVFLFPPKPKDTLMISRTPEVTCVVVDVSQEDPEVQFNWYVDGVEVHNAKTKPREEQFNSTYRVVSVLTVLHQDWLNGKEYKCKVSNKGLPSSIEKTISKAKGQPREPQVYTLPPSQEEMTKNQVSLTCLVKGFYPSDIAVEWESNGQPENNYKTTPPVLDSDGSFFLYSRLTVDKSRWQEGNVFSCSVMHEALHNHYTQKSLSLSLGK

SEQ ID NO: 76 - protein, 107 aa, synthetic construct [sequence omitted]

SEQ ID NO: 77 - protein, 106 aa, synthetic construct
GQPKAAPSVTLFPPSSEELQANKATLVCLISDFYPGAVTVAWKADSSPVKAGVETTTPSKQSNNKYAASSYLSLTPEQWKSHRSYSCQVTHEGSTVEKTVAPTECS

SEQ ID NO: 78 - protein, 168 aa, synthetic construct
RDGPAGSWEQLIQERRSHEVNPAAHLTGANSSLTGSGGPLLWETQLGLAFLRGLSYHDGALVVTKAGYYYIYSKVQLGGVGCPLGLASTITHGLYKRTPRYPEELELLVSQQSPCGRATSSSRVWWDSSFLGGVVHLEAGEEVVVRVLDERLVRLRDGTRSYFGAFMV

SEQ ID NO: 79 - protein, 196 aa, synthetic construct
HHHHHHHHHHGGGGSGGGGSGGGGSIEGRDGPAGSWEQLIQERRSHEVNPAAHLTGANSSLTGSGGPLLWETQLGLAFLRGLSYHDGALVVTKAGYYYIYSKVQLGGVGCPLGLASTITHGLYKRTPRYPEELELLVSQQSPCGRATSSSRVWWDSSFLGGVVHLEAGEEVVVRVLDERLVRLRDGTRSYFGAFMV

SEQ ID NO: 80 - protein, 412 aa, synthetic construct
DKTHTCPPCPAPELLGGPSVFLFPPKPKDTLMISRTPEVTCVVVDVSHEDPEVKFNWYVDGVEVHNAKTKPREEQYGSTYRVVSVLTVLHQDWLNGKEYKCKVSNKALPAPIEKTISKAKGQPREPQVYTLPPSREEMTKNQVSLTCLVKGFYPSDIAVEWESNGQPENNYKTTPPVLDSDGSFFLYSKLTVDKSRWQQGNVFSCSVMHEALHNHYTQKSLSLSPGGGGGSGGGGSGGGGSIEGRDGPAGSWEQLIQERRSHEVNPAAHLTGANSSLTGSGGPLLWETQLGLAFLRGLSYHDGALVVTKAGYYYIYSKVQLGGVGCPLGLASTITHGLYKRTPRYPEELELLVSQQSPCGRATSSSRVWWDSSFLGGVVHLEAGEEVVVRVLDERLVRLRDGTRSYFGAFMV

SEQ ID NO: 81 - protein, 196 aa, synthetic construct
HHHHHHHHHHGGGGSGGGGSGGGGSIEGRDGHGGSWEQLIQERRSHQNNPAAHLTGANSSLTGSGGPLLWETQLGLAFLRGLDYHDGALVANKAGYYYIYSKVQLGGVGCPLGLASTITHGLYKRTPRYPEELELLVSQQSPCGRATSNSRVWWDSSFLGGVVHLEVGEEVVVRVLDERLVRLRDGTRSYFGAFMV

SEQ ID NO: 82 - protein, 197 aa, synthetic construct
HHHHHHHHHHGGGGSGGGGSGGGGSIEGRDGGKGSWEKLIQDQRSHQANPAAHLTGANASLIGIGGPLLWETRLGLAFLRGLTYHDGALVTMEPGYYYVYSKVQLSGVGCPQGLANGLPITHGLYKRTSRYPKELELLVSRRSPCGRANSSRVWWDSSFLGGVVHLEAGEEVVVRVPGNRLVRPRDGTRSYFGAFMV

SEQ ID NO: 83 - protein, 15 aa, synthetic construct
KASQSVDFDGESYMN

SEQ ID NO: 84 - protein, 119 aa, synthetic construct
QVQLVQSGAEVKKPGASVKVSCKASGYTFIDHIMNWVRKAPGQGLEWMGRIYPVSGETNYNQKFMGRATFTVDRSTSTVYMELSSLRSEDTAVYYCGRGSYYWNAMDYWGQGTLVTVSS

SEQ ID NO: 85 - protein, 119 aa, synthetic construct
QVQLVQSGAEVKKPGASVKVSCKASGYTFIDHIMNWVRKAPGQGLEWIGRIYPVSGETNYNQKFMGRVTFTVDRSTSTVYMELSSLRSEDTAVYYCGRGSYYWNAMDYWGQGTLVTVSS

SEQ ID NO: 86 - protein, 111 aa, synthetic construct
EIVMTQSPATLSVSPGERATLSCKASQSVDFDGDSYMNWYQQKPGQPPRLLIYSASNLESGIPARFSGSGSGTEFTLTISSLQSEDFAVYYCQQSIEDPWTFGQGTKLEIK

SEQ ID NO: 87 - protein, 111 aa, synthetic construct
EIVMTQSPATLSVSPGERATLSCKASQSVDFDGDSYMNWYQQKPGQAPRLLIYSASNLESGIPARFSGSGSGTEFTLTISSLQSEDFAVYYCQQSIEDPWTFGQGTKVEIK

SEQ ID NO: 88 - protein, 111 aa, synthetic construct
DIVMTQSPDSLAVSLGERATINCKASQSVDFDGDSYMNWYQQKPGQPPKLLIYSASNLESGVPDRFSGSGSGTDFTLTISSLQAEDVAVYYCQQSIEDPWTFGQGTKVEIK

SEQ ID NO: 89 - protein, 111 aa, synthetic construct
EIVMTQSPATLSVSPGERATLSCKASQSVDFDGESYMNWYQQKPGQPPRLLIYSASNLESGIPARFSGSGSGTEFTLTISSLQSEDFAVYYCQQSIEDPWTFGQGTKLEIK

SEQ ID NO: 90 - protein, 111 aa, synthetic construct
EIVMTQSPATLSVSPGERATLSCKASQSVDFDGESYMNWYQQKPGQAPRLLIYSASNLESGIPARFSGSGSGTEFTLTISSLQSEDFAVYYCQQSIEDPWTFGQGTKVEIK

SEQ ID NO: 91 - protein, 111 aa, synthetic construct
DIVMTQSPDSLAVSLGERATINCKASQSVDFDGESYMNWYQQKPGQPPKLLIYSASNLESGVPDRFSGSGSGTDFTLTISSLQAEDVAVYYCQQSIEDPWTFGQGTKVEIK

SEQ ID NO: 92 - protein, 121 aa, synthetic construct
QVQLVQSGAEVKKPGASVKVSCKASGYTFTSYNVHWVRQAPGQGLEWIGAVYPGNGDTSYNQKFKGRATLTADKSTSTVYMELSSLRSEDTAVYYCARGSYYYTSSYFDHWGQGTLVTVSS

SEQ ID NO: 93 - protein, 121 aa, synthetic construct
QVQLVQSGAEVKKPGASVKVSCKASGYTFTSYNVHWVRQAPGQGLEWMGAVYPGNGDTSYNQKFKGRATLTADKSTSTAYMELSSLRSEDTAVYYCARGSYYYTSSYFDHWGQGTLVTVSS

SEQ ID NO: 94 - protein, 121 aa, synthetic construct
QVQLVQSGAEVKKPGASVKVSCKASGYTFTSYNVHWVRQAPGQGLEWIGAVYPGNGDTSYNQKFKGRATLTADKSTSTAYMELSSLRSEDTAVYYCARGSYYYTSSYFDHWGQGTLVTVSS

SEQ ID NO: 95 - protein, 111 aa, synthetic construct
EIVLTQSPATLSVSPGERATLSCKASQSVDFDGDSYMNWYQQKPGQPPRLLIYTASNLESGIPARFSGSGSGTEFTLTISSLQSEDFAVYYCQQSYEDPFTFGQGTKLEIK

SEQ ID NO: 96 - protein, 111 aa, synthetic construct
EIVMTQSPATLSVSPGERATLSCKASQSVDFDGDSYMNWYQQKPGQPPRLLIYTASNLESGIPARFSGSGSGTEFTLTISSLQSEDFAVYYCQQSYEDPFTFGQGTKLEIK

SEQ ID NO: 97 - protein, 111 aa, synthetic construct
EIVMTQSPATLSVSPGERATLSCKASQSVDFDGDSYMNWYQQKPGQAPRLLIYTASNLESGIPARFSGSGSGTEFTLTISSLQSEDFAVYYCQQSYEDPFTFGQGTKLEIK

SEQ ID NO: 98 - protein, 111 aa, synthetic construct
DIVLTQSPDSLAVSLGERATINCKASQSVDFDGDSYMNWYQQKPGQPPKLLIYTASNLESGIPDRFSGSGSGTDFTLTISSLQAEDVAVYYCQQSYEDPFTFGQGTKVEIK

SEQ ID NO: 99 - protein, 111 aa, synthetic construct
DIVMTQSPDSLAVSLGERATINCKASQSVDFDGDSYMNWYQQKPGQPPKLLIYTASNLESGVPDRFSGSGSGTDFTLTISSLQAEDVAVYYCQQSYEDPFTFGQGTKVEIK